European Patent Application EP 4 269 589 A1, published November 1, 2023. Title: PLANT ACIDIC INVERTASE ACTIVATOR MANUFACTURING METHOD, PLANT ACIDIC INVERTASE ACTIVATOR, AND PLANT ACIDIC INVERTASE ACTIVATION METHOD. Applicant: Panasonic Intellectual Property Management Co., Ltd. The sequence listing filed with the application follows.

SEQUENCE LISTING (22 sequences)

SEQ ID NO: 1 - protein, 630 aa, Synechocystis PCC6803
MLKLSWKSLLVSPAVIGAALVAGAASAAPDNVTNAQVLDQLDQYTAEGQSSAIDQVTSVSELRDVQPTAWAYEALKSLVERYGCIVGYPDRTFRGDRALSRWEFAAGLNACMNVMERLIQENVAVLREDIDKLKRLMQEFEAELAALGARVDNLEARTSFLEDHQFSTTTKLTGEVIFAPTAIFGTKKTLNNQTDNNQAVFQNRVRLQFNTSFSGEDLLVTRLAAGNGNRFKSFYPTQNVIDPETGNPIGIVGDYYESPTFTQVHQLSPGDNNNVAVDWLAYYVPLDLGENFRLNNYIAAWGGIWDDFVPTLNPYFDDYTGGKGSLSQFTAQNPIYSIGGGTGIGTSLELGFLSNLLGPTSLSLGYLASTGNNPSSGGSVTNPATGNNYDFSSGGNGLFNGGYSALAQITTNIFDRVSLGFTYVNAYTTPDAAIFGKGGTQGIVGTTAANLNRSELNDDFVNGLGVGAPPVDAATYNNNVSGGSTSGNVINPYDFGGKQTNSYGVQMAWNIADWLSFSAYGSYTNVTLIGKDNGDIWTYGGGFAFPDLGKEGNVLGIFAGVQPYVSGFTNNTLGTTFVTTANPLQVELFYKYQLTDNLSITPGVIWISKPEQTTNATDAFIGTVRGTFTF

SEQ ID NO: 2 - protein, 532 aa, Synechococcus sp. NIES-970
MSKAMRNLLSGATVALGATVAFSGAAIAEENQAVLDQISQYSTDNSVAQVNSVFQLSDVSPSDWAFDALRNLVENYNCIVGYPDGTFRGTRPLSRYEFAAGLNACLQQIERMLEGGGEVTQEDLAALRRLLNEFEAELATLGARVDDLDGRVEFLEDNQFSTTTKLNGEVIFNLGGAFGDSRADGPGPIDDEFTFSNRVRLNLDTSFTGRDRLRTRLEAGNITRLDRATGVDAARLGFDTNNGNDVEIGKLFYRFPVGDNITAYVGAVGLGLDDIFDVTNPYFESSGNGALSRFGRFNPIYRGPDGAGAGFNFDLGERVTFSAAYLADDGGASSPVSKNGLFNGNYTAGAQLDFAPSDNIMLSAVYTRRYQQGGDVNLSGSTGSDFAADPFGFAASSNNFGLQGSWLIGEKFNLGGWVGYTNADLKDPVVTGNADVWNWAVNAALLDVGGEGNTLGFIFGQPPKLTEADIDFGGGPITFDGSDSTYLAELQYRYKVNNNITITPGAYVLWNPNQNDANDTIVVGTVRTTFSF

SEQ ID NO: 3 - protein, 567 aa, Anabaena cylindrica PCC 7122
MSNLLWKSLVVSPAVLGAALLVSGTAIASPAAGNSASNAATEVSILETQAATEVVQQPVVLAQVKQDTQVLDQVKRYSNEGQNLQSQVTSVSQFSDVQPTDWAFQALQSLVERYGCIAGYPNGTYRGNRALTRYEFAAGLNACLDRVNELIATATADMVTKQDLATLQRLQEEFSAELATLRGRVDALEARTAELEANQFSTTTKLQGEAIFALTDAFNGDIAGKTVFQDRVRLNLQSSFTGRDMLNTRLAAGNAQNFGNTGESRQTFDVGSTGTNNVVLDKLTYEAPVGPAQVYIAATGGKHSHYAAVNNPYFFDKTDGGNGALSTFSSENPIYRIGGGSGIALNVPFGQGGGILKPSSLTLGYLASEANSPAAGEGLFDGNYAALGQLNFNVGNRIALAATYVHGYHGASSRLFDSGEGDDIVGTSLANNLSLGSASSSNSYGVSAAFRPSDKLSVSGFVSYHDITGFGAGDDYEAWSYGVGVALPDFGKKGNVLGIFGGAQPYSFNNNGGANSGDIPYQVEGFYKYRVSDNISVTPGVIWLPSIGQSSSSEDTFIGTLRTTFTF

SEQ ID NO: 4 - protein, 300 aa, Synechocystis PCC6803
MRVILCGYYGQDNAGDEALLVCLLQMLPATVEPVVLSANPQVTTARYGVKAHYNRDWGKIWQLLGQCDGFIWGGGSLMQDVTSVVSPLYYGGLMAIAQMRRLKTIAWAQGIGPLRRPPLRWFTQQVLRGCSGISVRDQASLQLVKQWGLKAFLAADPVWSLAAENASSSPSPLPMVAVNLRAHPLLTLERLAVITEALRDFQHQTQTHVRLIPLQKSQDLAIAEAIAVELPGSHEILYRPDPRECKGLFRGAEFTIGMRLHSLIMAAAEGSACFALSYDPKVSRLIAEVGLPGRELADLP

SEQ ID NO: 5 - protein, 339 aa, Synechocystis sp. PCC7942
MRALLCGYYGEGNGGDEALLAALLQLLPPTVEPLVLSGNPAATRTCYGVEACDRRSGAAVWQALRRSDLFIFGGGSLIQDVTSWTSPLYYCGLMGLAQQLGLKTIAWAQGIGPLQRKRTRWLARRTFQHCDRITVRDRGSAALLKEWGISVAIAPDPVWALEPLPLDQPLSNQEAIAVCLRPHPELTPERSDRLKAALTTLQSQTQAPILLIPFHHQQDRPLAAQWASEIPQAEVLDWQHPRQLLSYFQSVRLTIAMRFHGLVMAAAAGNRCFGLSYDPKVRRFLDALEQPGWDLPEIPDSAEAIAAAWLESWQAEPIHAAAIADLRQQVDVHRQALVF

SEQ ID NO: 6 - protein, 350 aa, Anabaena cylindrica PCC 7122
MVKIRALLSGYYGKGNGGDEALLATLLQMLPPDVTPVVLSGNPEETKKRYGVESYNRMAFLQIIKALRSCDAFIWGGGSLMQDATSSISPFYYGGLMALAQAMGLKTVAWGQGIGPLLRSQTRWLAKRNFALCTKISVRDRSSAALLSNWGIPHILAPDPVWALESKPVTELADLPKPRIAVILRNHPQLTETRLANLIHALVDLQQATQAFILLLPFQKSEDLDIAEKIQLQLKDVSKIICAEDPQLLKGIFRGVEMAIGMRLHSLIMAASEGCRCFALSYDPKVNHLMEDLEIPGWDLKDLPTDVDLMSKTWIQYYHNSEALSSEKIQSLVNGAFLHRDLLRASLSNK

SEQ ID NO: 7 - DNA, 1352 bp, Synechocystis PCC6803
atgcttaaactatcttggaagtccctgttagtgagccctgctgtgatcggtgccgcccttgtggctggtgctgctagtgctgctcccgacaacgttacgaatgctcaagttttagaccaattagaccaatacactgccgaaggtcagtcttctgccattgatcaagtaaccagcgttagcgaactccgcgatgtgcaacccactgcctgggcctatgaagcgctcaagagcttggtggaacgctacggttgtatcgttggttaccctgaccgtaccttccgtggtgatcgagccctcagccgttgggaatttgccgctggtcttaacgcctgtatgaacgttatggaacgtttgattcaggaaaacgtggctgttctccgggaggacatcgacaaactgaaacgcctcatgcaggaattcgaggcagaattggctgctttgggtgctcgggttgataacctcgaagcccgcacctctttcctcgaagaccatcagttttctaccaccaccaaattgaccggggaagtaatatttgctcccaccgccatttttggtaccaaaaagactctcaacaaccaaaccgataacaaccaagcggtattccagaaccgggttcgtttacagttcaacaccagcttctccggtgaagacctgttggtcactcgtctcgccgctggtaacggtaatcgcttcaagagcttctatcctactcagaatgttattgatcccgagaccggtaaccccatcggtattgtaggtgactactatgaaagccccacctttacccaggtgcaccagctttcccccggcgacaacaacaacgtagccgttgactggttagcttactatgttcccttggatctgggcgaaaacttccgtctcaacaactacattgctgcttggggcggtatctgggatgacttcgttcctaccctgaacccctatttcgacgactacactggcggcaaaggttccttgagtcagttcaccgcccagaaccccatctactccattggtggcggtactggtataggtacaagcctagagttgggcttcctcagcaatctgttgggccccacttccttgagcttgggttacttggctagcacgggcaacaaccccagcagtggtggttctgttactaaccctgccactggcaacaattatgacttcagcagcggtggtaacggtttgtttaacggtggctatagcgccttggctcaaattaccaccaacattttcgaccgggttagcctaggcttcacctacgttaatgcctacaccacccctgatgccgctatcttcggtaaaggtggcactcaaggtatcgtcggtaccactgcggctaacct

SEQ ID NO: 8 - DNA, 1353 bp, Synechococcus sp. NIES-970
atgtctaaagcaatgagaaatcttctcagtggtgcaaccgttgctctcggtgcaactgttgctttttctggcgcagcgatcgccgaagaaaaccaagccgtcctcgaccagatcagtcaatacagcactgataactccgttgctcaggtcaacagcgttttccagctcagcgacgtttccccttccgattgggcttttgacgcgctccgcaacttggttgaaaactacaactgtatcgttggttatcctgatggtactttccgtggcactcgccccctcagccgttatgagttcgccgcaggtctgaatgcttgtttgcaacagatcgaacggatgctcgaaggtggcggtgaagtaacccaagaagatctcgcagccctccgtcgtctgctcaacgaatttgaagcagaactagctaccctcggcgctcgtgttgatgaccttgatggccgtgttgagttccttgaagacaatcagttctccaccaccaccaaactgaatggggaagttatcttcaaccttggtggcgcttttggcgatagcagagctgatggtcctggcccaatcgatgatgagttcacattcagcaatcgtgttcgtctgaacctagacactagcttcactggtcgcgatcgcctccgcactcgtcttgaagctggcaatatcactcgcttagaccgtgcaactggtgtagatgcagcccgtctcggctttgacactaacaacggtaatgatgttgaaattgggaaattgttctaccgcttccctgtaggtgacaacattactgcctatgtcggtgccgttggcctaggtcttgatgacatatttgatgtaaccaacccatattttgagagcagcggtaatggtgccctctctcgtttcggtcgttttaaccccatctaccgtggccccgatggtgctggtgctggttttaacttcgatcttggtgaaagagttaccttctccgcagcttaccttgcggatgatggtggtgctagcagccctgtctcgaagaatggcctgttcaatggcaactacactgcgggtgctcagctcgattttgctccctctgacaacatcatgctgtctgccgtttatacccgtcgctaccaacagggtggcgatgtcaacctgagcggtagcactggtagtgattttgctgcagatccttttggttttgctgcttcttccaacaacttcggcttacaaggtagctggttgatcggtgaaaaattcaaccttggtggctgggtcggctacaccaatgctgatctcaaagatcctgttgtcaccggtaacgctgatgtttggaactgggctgttaacgccgctctacttgatgtcggcggcgaa

SEQ ID NO: 9 - DNA, 1360 bp, Anabaena cylindrica PCC 7122
atgtctaatctattgtggaaatccttggtggttagcccagccgtgttgggagccgccttattagtttcaggaacagcgatcgcatcgcccgccgcaggcaactcagcctcaaatgctgctactgaagtatcaatactagaaacacaagcggcaacagaggttgttcaacaacctgtagtattggctcaagtcaagcaagacactcaggttttagatcaagttaaacgctacagtaacgaaggtcaaaatctacaatctcaagtaacatcagtctctcagttttccgatgtccaaccaactgactgggcattccaagctttgcagtccttggtggaacgttatggttgtatcgcaggttatcccaatggtacatatcgcggaaaccgtgctttaacccgttatgaatttgccgctggtttgaatgcctgtttagaccgggtgaatgaattgattgccacagcaacagctgacatggtgacaaaacaggatttagccaccttacagcgcttgcaagaagaattttctgctgaattggcaactttacgcggtcgtgtcgatgctttggaagcacgcactgctgagttagaagctaatcaattctctactaccaccaaattgcaaggtgaagctatttttgctctgaccgatgcttttaatggtgacattgccggtaagaccgtttttcaagatagagtgcgtttgaacctgcaaagcagcttcacaggtcgagatatgttgaatacccgtttggctgcgggtaatgcacaaaactttggaaacactggggaaagtagacaaacctttgacgttggtagcactgggactaacaatgttgtgttagacaaactgacctatgaagctcctgttggtccagcacaggtctacatagcagctacaggtggtaaacacagccattatgctgctgttaacaacccttacttctttgataaaactgatggtggtaacggtgctttaagtacctttagttctgaaaaccccatctatcgaattggtggtggttctggtattgcccttaatgtaccctttggtcaaggtggcggtattctcaaaccaagttcattgacattgggttatttggcttctgaggctaatagtcctgctgctggtgaaggtttgttcgacggtaactatgctgctttaggtcagttaaactttaacgttggtaatcgcattgccttagctgctacttatgtacatggttatcatggtgctagtagccgtttgtttgactcaggagagggtgatgatatcgtaggtacatcactagctaataatctcagtttaggtagcgcctcgtccagcaactcctacggtgtttctgctgccttcagacctagcg

SEQ ID NO: 10 - DNA, 1032 bp, Synechocystis PCC6803
atgcgtgtcattctgtgtggttactacggccaagacaatgctggggatgaagcccttttagtctgtttgctgcaaatgcttcctgcgacggtggagccagtggtgctctccgccaatccccaggtcaccacagcgagatacggtgttaaagcccactacaaccgagactggggcaaaatttggcagcttttgggtcaatgtgacggttttatctgggggggaggcagtttgatgcaggatgtgaccagcgtggttagtcccctatactacggtggtttgatggcgatcgcccagatgcggcgtttaaaaaccattgcctgggcccagggcattggcccccttagaaggccgccgttgcgctggtttacccaacaggtgctccggggttgtagcggcatcagcgtacgggatcaagcttctttgcaattagttaaacaatggggcttaaaggcttttttagcggcggatccggtgtggtctttagccgctgaaaatgcgtcttcttcccccagccctttgcccatggtggcggtgaatttgcgggcccatcctttgttaaccttggaacgcttggcggtcattaccgaagccctaagggattttcaacaccagacccaaacccatgtgcggctcattcccctacaaaaatcccaggatttggccattgccgaagcgatcgccgtggaattgccggggagtcatgaaattctttaccgccccgaccccagggaatgtaaaggtttgttccggggggcggaattcaccattggcatgcggctccacagtttaatcatggccgcggcggagggcagtgcctgctttgcccttagttatgaccctaaagttagtcgtttaatcgcagaggtgggactaccgggccgggaattggcggatttacccagggatagcaacgaactcagccaggtttggcagggacatttccggcaaagacaaccctctaccggggtagagttcttgcaaaaatctgcccttcagcatcaaactttgttgcagaaaatttttgttgactag

SEQ ID NO: 11 - DNA, 1020 bp, Synechocystis sp. PCC7942
atgcgggcgttgctctgtggctattacggagagggcaatgggggagatgaggcgctgttggcagcgctgttgcaactcttgccgccgacagtggaaccgctggtgctgtcggggaatcctgcggcaactcgcacttgctacggcgtagaagcttgcgatcgccgatcgggggctgcggtttggcaggcactgcgacgcagtgatctattcatctttggcggcggcagcctgattcaagatgtcacaagctggacgagccctctctactactgcggtctgatggggctggcacaacagttaggtctcaaaacgatcgcctgggcccagggcattgggccactgcagcgcaaacgaacccgctggttggcacgccgaacgtttcagcactgcgatcgcattacagtgcgcgatcgcggttctgctgccttgctaaaagagtgggggatttctgtggcgattgccccggatcccgtttgggctttagagccgctgcctttagatcagccgctgtcgaaccaagaggcgatcgcggtttgtctgcggccccaccctgagttgacgcctgagcgcagcgatcgcttgaaagctgccctgacaactctgcaatcgcaaacccaagcacccatcctgctgattcccttccaccaccagcaagatcgaccactggccgcgcaatgggcaagcgaaattccccaagcagaagttttggactggcagcatccgcgccagctcctcagctactttcagtcggtgcgattaacgatcgccatgcgcttccatggattagtgatggcagcagcggctggaaatcgttgctttggcctcagctatgaccccaaagtgcgccgtttcctggatgcccttgagcaacccggctgggatttgccggagattccagactctgctgaggcgatcgcggccgcttggttagagtcttggcaagcagaaccgattcatgccgctgcgatcgcggacctccgtcagcaagtggatgtccatcgccaggctttagttttttga

SEQ ID NO: 12 - DNA, 1053 bp, Anabaena cylindrica PCC 7122
ctacttattactcaatgatgctctcaataaatcccgatgtaaaaaagctccatttactaaagattgtattttctcagatgataatgcttcgctattgtgataatattgaatccaggttttactcattaaatctacatcagttggtaaatcctttaaatcccatccaggtatttctaaatcttccatcaaatggttaaccttggggtcataactcaaagcaaaacaacgacaaccttcactagctgccataattaaactgtgtagacgcatccctattgccatttctacaccacgaaatataccttttaaaagttgtggatcttctgcacagataattttactaacatcttttaattgcagttgaattttttctgcaatatctaaatcttcacttttttgaaaaggcaataataaaataaatgcttgggtagcttgttgtaaatcaactaaggcatggattaaatttgctaaccgagtttctgtaagttggggatgatttcttaaaataacggcaattctaggttttggtaaatctgctaattctgttactggtttagattctaaagcccaaactggatcaggtgcaagaatatgaggtatgccccaatttgataataaagccgcactagagcgatcgcgtacactgattttagtacaaagagcaaaatttcgctttgctaaccaacgagtttgcgatcgcaataaaggccctattccctgtccccaagctacagttttcaaacccatcgcttgagctaaagccattaatcccccataataaaaagggctaatgctgctagtcgcatcctgcattaaacttccaccaccccagatgaaagcatcacaggaacgcaaagctttgataatctgcaaaaacgccatacggttgtaactttccacaccataacgctttttagtttcctcaggattcccagaaagcaccacaggcgttacatcaggtggtagcatttgcagaagtgtcgccaacaaagcttcatcaccaccattacctttaccgtaatacccagacaataacgcccgtatcttcaccat

SEQ ID NO: 13 - DNA, 40 bp, Artificial Sequence
  Synthesized Primer
cagtgaattcgagctcggtatatagcgttgcagtccctgg

SEQ ID NO: 14 - DNA, 40 bp, Artificial Sequence
  Synthesized Primer
gattacgccaagcttgcatgaccgcggtcacttcataacc

SEQ ID NO: 15 - DNA, 47 bp, Artificial Sequence
  Synthesized Primer
cagtgaattcgagctcggtaataaccgttgtcccttttgtttcatcg

SEQ ID NO: 16 - DNA, 45 bp, Artificial Sequence
  Synthesized Primer
tgttagtgagccctgctgttagctcccagtatctctatcactgat

SEQ ID NO: 17 - DNA, 51 bp, Artificial Sequence
  Synthesized Primer
acagcagggctcactaacagttttagagctagaaatagcaagttaaaataa

SEQ ID NO: 18 - DNA, 44 bp, Artificial Sequence
  Synthesized Primer
gattacgccaagcttgcatggggaacaagctgaatctgggcatc

SEQ ID NO: 19 - DNA, 45 bp, Artificial Sequence
  Synthesized Primer
ttttagtctgtttgctgcatagctcccagtatctctatcactgat

SEQ ID NO: 20 - DNA, 51 bp, Artificial Sequence
  Synthesized Primer
tgcagcaaacagactaaaagttttagagctagaaatagcaagttaaaataa

SEQ ID NO: 21 - DNA, 19 bp, Synechocystis PCC6803
acagcagggctcactaaca

SEQ ID NO: 22 - DNA, 19 bp, Synechocystis PCC6803
tgcagcaaacagactaaaa